European Patent Application EP 4 302 774 A1, published January 10, 2024. Title: USE OF ENHANCED TBX1 EXPRESSION IN REPAIRING HEART TISSUE INJURY. Applicant: SHANGHAI CHILDREN' S MEDICAL CENTER, SHANGHAI JIAOTONG UNIVERSITY SCHOOL OF MEDICINE. The sequence listing filed with the application follows.

SEQUENCE LISTING (2 sequences)

SEQ ID NO: 1 - DNA, 1488 bp, Homo sapiens
atgcacttcagcaccgtcaccagggacatggaagccttcacggccagcagcctgagcagcctgggggccgcggggggcttcccgggcgccgcgtcgcccggcgccgacccgtacggcccgcgcgagcccccgccgccgccgccgcgctacgacccgtgcgccgccgccgcccccggcgccccgggcccgccgccgccgccgcacgcctacccgtttgcgccggccgccggggccgccaccagcgccgccgccgagcccgagggccccggggccagctgcgcggccgcagccaaggcgccggtgaagaagaacgcgaaggtggccggtgtgagcgtgcagctagagatgaaggcgctgtgggacgagttcaaccagctgggcaccgagatgatcgtcaccaaggccggcaggcggatgtttcccaccttccaagtgaagctcttcggcatggatcccatggccgactatatgctgctcatggacttcgtgccggtggacgataagcgctaccggtacgccttccacagctcctcctggctggtggcggggaaggccgaccctgccacgccaggccgcgtgcactaccacccggactcgcctgccaagggcgcgcagtggatgaagcaaatcgtgtccttcgacaagctcaagctgaccaacaacctactggacgacaacggccacattattctgaattccatgcacagataccagccccgcttccacgtggtctatgtggacccacgcaaagatagcgagaaatatgccgaggagaacttcaaaacctttgtgttcgaggagacacgattcaccgcggtcactgcctaccagaaccatcggatcacgcagctcaagattgccagcaatcccttcgcgaaaggcttccgggactgtgaccctgaggactggccccggaaccaccggcccggcgcactgccgctcatgagcgccttcgcgcgctcgcggaaccccgtggcttccccgacgcagcccagcggcacggagaaagacgcggctgaggcccggcgagaattccagcgcgacgcgggcgggccagcagtgctcggggacccggcgcatcctccgcagctgctggcccgggtgctaagcccctcgctgcccggggccggcggcgccggcggcttagtcccgctgcccggcgcgcccggaggccggcccagtcccccgaaccccgagctgcgcctggaggcgcccggcgcatcggagccgctgcaccaccacccctacaaatatccggccgccgcctacgaccactatctcggggccaagagccggccggcgccctacccgctgcccggcctgcgtggccacggctaccacccgcacgcgcatccgcaccaccaccaccaccccgtgagtccagccgccgcggccgccgccgccgctgccgcagctgccgcggccgccaacatgtactcgtcggccggagccgcgccgcccggctcctacgactattgccccagataa

SEQ ID NO: 2 - DNA, 1467 bp, Mus musculus
atgatctccgccgtgtctagtccgtggctcacgcagctctcgcacttctgcgacgttgcagccttcgcagccagcagtctgagcggcctgggatccccgtcgcctggcgccgacccgttcggccctcgcgagccgccgccaccgcgctacgatccgtgcgctgcagtccccggtgccccgggcccgccgccgccgcgcgcctatcctttcgcgcccgcccccggggcggctggcagctcggcggcggagtccgagggtccgggggctagccgcgcggctgcggtcaaggctccggtgaagaagaacccgaaggtggccagcgtgagcgtgcagctggagatgaaggcgctgtgggacgagttcaatcagctgggcaccgagatgatcgtcaccaaggcaggcagacgaatgttccccacgttccaagtgaagctttttggaatggatcccatggccgactacatgctgctcatggactttgtgcccgtagatgacaagcgctaccggtatgctttccatagctcctcctggctggtggccggcaaggcagatcctgctacacctggccgagtacactaccacccggactcgccggctaagggcgcacagtggatgaaacagattgtgtctttcgacaagctgaaactgaccaataacctgctggatgacaatggccatattattctcaactccatgcacagatatcagccccgattccatgttgtctatgtggaccctcgaaaagacagtgagaaatatgcagaggagaacttcaaaacttttgtgtttgaggagacacgcttcactgcagtcactgcctaccagaatcaccggatcacgcagcttaagattgccagcaaccccttcgccaaaggcttccgggattgcgacccggaggactggccccggaaccaccggcccggagcgctgccgctcgtgagtgcctttgctcgctctcggaatcccgtggcttcccccacgcagcccaatggctcagacaaagacgctgcagaagcccggcgcgagttcgaccgtgactccggacccgcagcgctcggcgacgctacgcacccgccgcagctgctggcgcgcgtgctgagccccgcactgcccgggcctggcggcctcgtcccgctacccggcggatccggaggccgccacagtcccccgcacgccgatctgcgcctggaggcgccgggcgcgtccgagccgctgcaccaccatccctacaagtacccggccgccgcctacgaccactacctcggggccaagagccggccggcgccctacccgctgccaggcctgcgcggccacggctaccacccgcacgcgcacccgcacgcgcacccgcaccatcaccaccaccccgcggtgaacccggccgccgccgccgctgctgccgcagcagccaacgtgtactcgtcggcggccgcgccgcccggtgcctacgactactgccccagatag